European Patent Application EP 4 714 463 A1, published March 25, 2026. Title: Formulacion para la inmunizacion de cerdos por la via oral. Applicant: CENTRO DE INGENIERIA GENETICA Y BIOTECNOLOGIA. Application CU. The sequence listing filed with the application follows.

SEQUENCE LISTING (3 sequences)

SEQ ID NO: 1 - protein, 624 aa, VPPA-Cerdo
MKRGLCCVLLLCGAVFVSPSQEIHARFRRGARSKVLRGQVVQGVIWLLLVTGAQGRLACKEDFRYAISSTNEIGLLGAEGLTTTWKDYDHNLQLDDGTIKAICTAGSFKVIALNVVSRRYLASLHKGLPTSVTFELLFDGTSPSIEEMGDDFGFGLCPFDSPVVKGRYNTTLLNGSAFYLVCPIGWTGVIECTAVSPTTLRTEVVKTFRREKPFPHRKDCVTTTVENEDLFYCRLGGNWTCVKGEPVIYTGGLKQCRWCGFDFNEPDGLPHYPIGKCILANETGYRIDSTDCNRNGVVISTEGSHECLIGNTSVKVHALDERLGPMPCRPKEIVSSEGPVRKTSCTFNYTKTLRNKYYEPRDSYFQQYMLKGEYQYWFDDVTDHHSDYFTEDIHHHHHHSNSGGGSGGGGSGGGGSKIEDERNLHEDFVFIKTIQRCKQGEGSLSLLNCEEIRSQFEDLVKGIMQSKEVKKKEKSFEMHKGDQDPQIAAHVISEASSKTASVLQWAKGYYTLSTNLVTLENGRQLAVKRQGIYYIYAQVTFCSRDAAGQAPFIASLCLRSPSGSERILLRAANTHSSSKPCGQQSIHLGGVFELQPGASVFVNVTDPSQVSHGTGFTSFGLLKL

SEQ ID NO: 2 - protein, 561 aa, VPPA-CHOK1
MASGGAFCLIANDGKADKIILAQDLLNSRISNIKNVNKSYGKPDPEPTLSQIEETHLVHFNAHFKPYVPVGFEYNKVRPHTGTPTLGNKLTFGIPQYGDFFHDMVGHHILGACHSSWQDAPIQGTSQMGAHGQLQTFPRNGYDWDNQTPLEGAVYTLVDPFGRPIVPGTKNAYRNLVYYCEYPGERLYENVRFDVNGNSLDEYSSDVTTLVRKFCIPGDKMTGYKHLVGQEVSVEGTSGPLLCNIHDLHKPHQSKPILLVTDENDTQRTCSHTNPKFLSQHFPENSHNIQTAGKQDITPITDATYLDIRRNVHYSCNGPQTPKYYQDIHHHHHHSNSGGGSGGGGSGGGGSKIEDERNLHEDFVFIKTIQRCKQGEGSLSLLNCEEIRSQFEDLVKGIMQSKEVKKKEKSFEMHKGDQDPQIAAHVISEASSKTASVLQWAPKGYYTLSTNLVTLENGRQLAVKRQGIYYIYAQVTFCSNRDAAGQAPFIASLCLRSPSGSERILLRAANTHSSSKPCGQQSIHLGGVFELQPGASVFVNVTDPSQVSHGTGFTSFGLLKL

SEQ ID NO: 3 - protein, 436 aa, VPPA-CHOK1
MDFILNISMKMEVIFKTDLRSSSQVVFHAGSLYNWFSVEIINSGRIVTTAIKTLLSTVKYDIVKSARIYAGQGYTEHQAQEEWNMILHVLFEEETESSASSENIHEKNDNETNECTSSFETLFEQEPSSEVPKDSKLYMLAQKTVQHIEQYGKAPDFNKVIRAHNFIQTIYGTPLKEEEKEVVRLMVIKLLKKISFYLTYIDIHHHHHHSNSGGGSGGGGSGGGGSKIEDERNLHEDFVFIKTIQRCKQGEGSLSLLNCEEIRSQFEDLVKGIMQSKEVKKKEKSFEMHKGDQDPQIAAHVISEASSKTASVLQWAPKGYYTLSTNLVTLENGRQLAVKRQGIYYIYAQVTFCSNRDAAGQAPFIASLCLRSPSGSERILLRAANTHSSSKPCGQQSIHLGGVFELQPGASVFVNVTDPSQVSHGTGFTSFGLLKL